European Patent Application EP 4 372 100 A1, published May 22, 2024. Title: Data analysis method for multiplex digital PCR using color-combination. Applicant: STILLA TECHNOLOGIES. The sequence listing filed with the application follows.

SEQUENCE LISTING (102 sequences)

SEQ ID NO: 1 - DNA, 19 bp, synthetic construct
  source 1..19: mol_type = other DNA
tctttccaagcaacagcag

SEQ ID NO: 2 - DNA, 20 bp, synthetic construct
  source 1..20: mol_type = other DNA
aatactgaccagccgtttga

SEQ ID NO: 3 - DNA, 22 bp, synthetic construct
  source 1..22: mol_type = other DNA
tccgagattatgcgccaaatgc

SEQ ID NO: 4 - DNA, 22 bp, synthetic construct
  source 1..22: mol_type = other DNA
tccgagattatgcgccaaatgc

SEQ ID NO: 5 - DNA, 21 bp, synthetic construct
  source 1..21: mol_type = other DNA
ctgtacagcatgaagtgcaag

SEQ ID NO: 6 - DNA, 15 bp, synthetic construct
  source 1..15: mol_type = other DNA
gcatgtaggcggtgg

SEQ ID NO: 7 - DNA, 19 bp, synthetic construct
  source 1..19: mol_type = other DNA
tgcccccctatgacctgct

SEQ ID NO: 8 - DNA, 19 bp, synthetic construct
  source 1..19: mol_type = other DNA
tgcccccctatgacctgct

SEQ ID NO: 9 - DNA, 20 bp, synthetic construct
  source 1..20: mol_type = other DNA
gccattgtttctctgtggag

SEQ ID NO: 10 - DNA, 20 bp, synthetic construct
  source 1..20: mol_type = other DNA
tcacggttcagttgttcacc

SEQ ID NO: 11 - DNA, 18 bp, synthetic construct
  source 1..18: mol_type = other DNA
tgattgcccgtctccgct

SEQ ID NO: 12 - DNA, 20 bp, synthetic construct
  source 1..20: mol_type = other DNA
actgattgcccgtctccgct

SEQ ID NO: 13 - DNA, 21 bp, synthetic construct
  source 1..21: mol_type = other DNA
cgttgatgcaatttctatgcg

SEQ ID NO: 14 - DNA, 20 bp, synthetic construct
  source 1..20: mol_type = other DNA
tcgatagtggctccaagtag

SEQ ID NO: 15 - DNA, 21 bp, synthetic construct
  source 1..21: mol_type = other DNA
cgcccagtcctgctcgcttcg

SEQ ID NO: 16 - DNA, 21 bp, synthetic construct
  source 1..21: mol_type = other DNA
cgcccagtcctgctcgcttcg

SEQ ID NO: 17 - DNA, 25 bp, synthetic construct
  source 1..25: mol_type = other DNA
tgaaacatacgttcccaaagagttt

SEQ ID NO: 18 - DNA, 26 bp, synthetic construct
  source 1..26: mol_type = other DNA
ctctccttctcagaaagtgtgcatat

SEQ ID NO: 19 - DNA, 25 bp, synthetic construct
  source 1..25: mol_type = other DNA
tgctgaaacattcaccttccatgca

SEQ ID NO: 20 - DNA, 25 bp, synthetic construct
  source 1..25: mol_type = other DNA
tgctgaaacattcaccttccatgca

SEQ ID NO: 21 - DNA, 18 bp, synthetic construct
  source 1..18: mol_type = other DNA
cctgcaggtcgactctag

SEQ ID NO: 22 - DNA, 21 bp, synthetic construct
  source 1..21: mol_type = other DNA
tgagcggataacaatttcaca

SEQ ID NO: 23 - DNA, 21 bp, synthetic construct
  source 1..21: mol_type = other DNA
cccgggtaccgagctcgaatt

SEQ ID NO: 24 - DNA, 21 bp, synthetic construct
  source 1..21: mol_type = other DNA
cccgggtaccgagctcgaatt

SEQ ID NO: 25 - DNA, 40 bp, synthetic construct
  source 1..40: mol_type = other DNA
gtctcggtactctctccgagattatgcgccaaatgcttac

SEQ ID NO: 26 - DNA, 34 bp, synthetic construct
  source 1..34: mol_type = other DNA
ctcggtactctctgactgattgcccgtctccgct

SEQ ID NO: 27 - DNA, 35 bp, synthetic construct
  source 1..35: mol_type = other DNA
tcggtactctctgacccgggtaccgagctcgaatt

SEQ ID NO: 28 - DNA, 32 bp, synthetic construct
  source 1..32: mol_type = other DNA
cgtgtgactgatactgattgcccgtctccgct

SEQ ID NO: 29 - DNA, 34 bp, synthetic construct
  source 1..34: mol_type = other DNA
cgtgtgactgatacgcccagtcctgctcgcttcg

SEQ ID NO: 30 - DNA, 32 bp, synthetic construct
  source 1..32: mol_type = other DNA
gtgtgactgatactgcccccctatgacctgct

SEQ ID NO: 31 - DNA, 31 bp, synthetic construct
  source 1..31: mol_type = other DNA
tcctgcctgccccgggtaccgagctcgaatt

SEQ ID NO: 32 - DNA, 31 bp, synthetic construct
  source 1..31: mol_type = other DNA
tcctgcctgccgcccagtcctgctcgcttcg

SEQ ID NO: 33 - DNA, 35 bp, synthetic construct
  source 1..35: mol_type = other DNA
ctgcctgccgtgctgaaacattcaccttccatgca

SEQ ID NO: 34 - DNA, 29 bp, synthetic construct
  source 1..29: mol_type = other DNA
ctccgaccggtgcccccctatgacctgct

SEQ ID NO: 35 - DNA, 36 bp, synthetic construct
  source 1..36: mol_type = other DNA
ctccgaccggtccgagattatgcgccaaatgcttac

SEQ ID NO: 36 - DNA, 35 bp, synthetic construct
  source 1..35: mol_type = other DNA
ctccgaccggtgctgaaacattcaccttccatgca

SEQ ID NO: 37 - DNA, 20 bp, synthetic construct
  source 1..20: mol_type = other DNA
ataatctcggagagagtacc

SEQ ID NO: 38 - DNA, 18 bp, synthetic construct
  source 1..18: mol_type = other DNA
ggcaatcagtcagagagt

SEQ ID NO: 39 - DNA, 15 bp, synthetic construct
  source 1..15: mol_type = other DNA
tacccgggtcagaga

SEQ ID NO: 40 - DNA, 18 bp, synthetic construct
  source 1..18: mol_type = other DNA
ggcaatcagtatcagtca

SEQ ID NO: 41 - DNA, 16 bp, synthetic construct
  source 1..16: mol_type = other DNA
gactgggcgtatcagt

SEQ ID NO: 42 - DNA, 14 bp, synthetic construct
  source 1..14: mol_type = other DNA
gggcagtatcagtc

SEQ ID NO: 43 - DNA, 11 bp, synthetic construct
  source 1..11: mol_type = other DNA
cccggggcagg

SEQ ID NO: 44 - DNA, 11 bp, synthetic construct
  source 1..11: mol_type = other DNA
tgggcggcagg

SEQ ID NO: 45 - DNA, 16 bp, synthetic construct
  source 1..16: mol_type = other DNA
gaatgtttcagcacgg

SEQ ID NO: 46 - DNA, 11 bp, synthetic construct
  source 1..11: mol_type = other DNA
ggggcaccggt

SEQ ID NO: 47 - DNA, 14 bp, synthetic construct
  source 1..14: mol_type = other DNA
atctcggaccggtc

SEQ ID NO: 48 - DNA, 13 bp, synthetic construct
  source 1..13: mol_type = other DNA
ttcagcaccggtc

SEQ ID NO: 49 - DNA, 48 bp, synthetic construct
  source 1..48: mol_type = other DNA
ctcatcgccaagaatagacagtcagagagtaccgagacaggcgatgag

SEQ ID NO: 50 - DNA, 46 bp, synthetic construct
  source 1..46: mol_type = other DNA
cctagcccagacaagaagagaacagtatcagtcacacggggctagg

SEQ ID NO: 51 - DNA, 50 bp, synthetic construct
  source 1..50: mol_type = other DNA
ccgcgccaggcacgaccacaggtgagcacggcaggcaggagggggcgcgg

SEQ ID NO: 52 - DNA, 47 bp, synthetic construct
  source 1..47: mol_type = other DNA
cggcgccagcggacgaggctgtgcaccggtcggaggtgggggcgccg

SEQ ID NO: 53 - DNA, 40 bp, synthetic construct; identical to SEQ ID NO: 25
  source 1..40: mol_type = other DNA

SEQ ID NO: 54 - DNA, 35 bp, synthetic construct
  source 1..35: mol_type = other DNA
actctctcttggtctactgattgcccgtctccgct

SEQ ID NO: 55 - DNA, 35 bp, synthetic construct
  source 1..35: mol_type = other DNA
tctcggtactctctcccgggtaccgagctcgaatt

SEQ ID NO: 56 - DNA, 34 bp, synthetic construct
  source 1..34: mol_type = other DNA
agctgcgttgtatcccgggtaccgagctcgaatt

SEQ ID NO: 57 - DNA, 34 bp, synthetic construct
  source 1..34: mol_type = other DNA
agctgcgttgtatcgcccagtcctgctcgcttcg

SEQ ID NO: 58 - DNA, 39 bp, synthetic construct
  source 1..39: mol_type = other DNA
ctagctgcgttgtatgctgaaacattcaccttccatgca

SEQ ID NO: 59 - DNA, 32 bp, synthetic construct
  source 1..32: mol_type = other DNA
gttggatcgatggtgcccccctatgacctgct

SEQ ID NO: 60 - DNA, 39 bp, synthetic construct
  source 1..39: mol_type = other DNA
gttggatcgatggtccgagattatgcgccaaatgcttac

SEQ ID NO: 61 - DNA, 38 bp, synthetic construct
  source 1..38: mol_type = other DNA
gttggatcgatggtgctgaaacattcaccttccatgca

SEQ ID NO: 62 - DNA, 34 bp, synthetic construct
  source 1..34: mol_type = other DNA
gtacgattgtggtgactgattgcccgtctccgct

SEQ ID NO: 63 - DNA, 34 bp, synthetic construct
  source 1..34: mol_type = other DNA
cgattgtggtgagcgcccagtcctgctcgcttcg

SEQ ID NO: 64 - DNA, 32 bp, synthetic construct
  source 1..32: mol_type = other DNA
gattgtggtgagctgcccccctatgacctgct

SEQ ID NO: 65 - DNA, 48 bp, synthetic construct
  source 1..48: mol_type = other DNA
atcgcccaagaatagacagaagaatagaccaagagagagtaccgagac

SEQ ID NO: 66 - DNA, 46 bp, synthetic construct
  source 1..46: mol_type = other DNA
acattgacattggacattcagacagatagatacaacgcagctagga

SEQ ID NO: 67 - DNA, 46 bp, synthetic construct
  source 1..46: mol_type = other DNA
cgtattgattcatcttctctcctacactgtaccatcgatccaacta

SEQ ID NO: 68 - DNA, 45 bp, synthetic construct
  source 1..45: mol_type = other DNA
tccattgataaccttctaatactacagctcaccacaatcgtacta

SEQ ID NO: 69 - DNA, 14 bp, synthetic construct
  source 1..14: mol_type = other DNA
tattcttgggcgat

SEQ ID NO: 70 - DNA, 14 bp, synthetic construct
  source 1..14: mol_type = other DNA
tccaatgtcaatgt

SEQ ID NO: 71 - DNA, 16 bp, synthetic construct
  source 1..16: mol_type = other DNA
aagatgaatcaatacg

SEQ ID NO: 72 - DNA, 15 bp, synthetic construct
  source 1..15: mol_type = other DNA
aaggttatcaatgga

SEQ ID NO: 73 - DNA, 22 bp, synthetic construct
  source 1..22: mol_type = other DNA
tccgagattatgcgccaaatgc

SEQ ID NO: 74 - DNA, 22 bp, synthetic construct
  source 1..22: mol_type = other DNA
tccgagattatgcgccaaatgc

SEQ ID NO: 75 - DNA, 19 bp, synthetic construct
  source 1..19: mol_type = other DNA
tgcccccctatgacctgct

SEQ ID NO: 76 - DNA, 25 bp, synthetic construct
  source 1..25: mol_type = other DNA
tgctgaaacattcaccttccatgca

SEQ ID NO: 77 - DNA, 19 bp, synthetic construct
  source 1..19: mol_type = other DNA
tgcccccctatgacctgct

SEQ ID NO: 78 - DNA, 19 bp, synthetic construct
  source 1..19: mol_type = other DNA
tgcccccctatgacctgct

SEQ ID NO: 79 - DNA, 21 bp, synthetic construct
  source 1..21: mol_type = other DNA
cgcccagtcctgctcgcttcg

SEQ ID NO: 80 - DNA, 25 bp, synthetic construct
  source 1..25: mol_type = other DNA
tgctgaaacattcaccttccatgca

SEQ ID NO: 81 - DNA, 25 bp, synthetic construct
  source 1..25: mol_type = other DNA
tgctgaaacattcaccttccatgca

SEQ ID NO: 82 - DNA, 21 bp, synthetic construct
  source 1..21: mol_type = other DNA
cccgggtaccgagctcgaatt

SEQ ID NO: 83 - DNA, 21 bp, synthetic construct
  source 1..21: mol_type = other DNA
cccgggtaccgagctcgaatt

SEQ ID NO: 84 - DNA, 23 bp, synthetic construct
  source 1..23: mol_type = other DNA
tcctatcctgagtagtggtaatc

SEQ ID NO: 85 - DNA, 20 bp, synthetic construct
  source 1..20: mol_type = other DNA
cctttcttgcggagattctc

SEQ ID NO: 86 - DNA, 18 bp, synthetic construct
  source 1..18: mol_type = other DNA
tgcgccagtctctcccag

SEQ ID NO: 87 - DNA, 18 bp, synthetic construct
  source 1..18: mol_type = other DNA
tgcgccagtctctcccag

SEQ ID NO: 88 - DNA, 22 bp, synthetic construct
  source 1..22: mol_type = other DNA
caccatccactacaactacatg

SEQ ID NO: 89 - DNA, 18 bp, synthetic construct
  source 1..18: mol_type = other DNA
tcctgacctggagtcttc

SEQ ID NO: 90 - DNA, 19 bp, synthetic construct
  source 1..19: mol_type = other DNA
catgaaccggaggcccatc

SEQ ID NO: 91 - DNA, 19 bp, synthetic construct
  source 1..19: mol_type = other DNA
catgaaccggaggcccatc

SEQ ID NO: 92 - DNA, 19 bp, synthetic construct
  source 1..19: mol_type = other DNA
gtggataaggtcatcacca

SEQ ID NO: 93 - DNA, 19 bp, synthetic construct
  source 1..19: mol_type = other DNA
caaggtgcttaggaactcg

SEQ ID NO: 94 - DNA, 23 bp, synthetic construct
  source 1..23: mol_type = other DNA
acgtccctcattctctatgtgcc

SEQ ID NO: 95 - DNA, 23 bp, synthetic construct
  source 1..23: mol_type = other DNA
acgtccctcattctctatgtgcc

SEQ ID NO: 96 - DNA, 20 bp, synthetic construct
  source 1..20: mol_type = other DNA
tggatttgaccctccatgat

SEQ ID NO: 97 - DNA, 20 bp, synthetic construct
  source 1..20: mol_type = other DNA
ccagacgagaccaatcatca

SEQ ID NO: 98 - DNA, 17 bp, synthetic construct
  source 1..17: mol_type = other DNA
  modified_base 2: mod_base = OTHER; note = locked nucleic acid LNA
  modified_base 5: mod_base = OTHER; note = locked nucleic acid LNA
  modified_base 6: mod_base = OTHER; note = locked nucleic acid LNA
ttctagaatgtgcctgg

SEQ ID NO: 99 - DNA, 17 bp, synthetic construct
  source 1..17: mol_type = other DNA
ttctagaatgtgcctgg

SEQ ID NO: 100 - DNA, 23 bp, synthetic construct
  source 1..23: mol_type = other DNA
gtgagaaagttaaaattcccgtc

SEQ ID NO: 101 - DNA, 20 bp, synthetic construct
  source 1..20: mol_type = other DNA
ccacacagcaaagcagaaac

SEQ ID NO: 102 - DNA, 24 bp, synthetic construct
  source 1..24: mol_type = other DNA
cacatcgaggatttccttgttggc